European Patent Application EP 4 707 298 A2, published March 11, 2026. Title: Human anti-FGF2 monoclonal antibody (MAB), pharmaceutical composition comprising the same, use thereof, and kit for cancer detection in a biological sample comprising said MAB. Applicant: INSTITUTO BUTANTAN. The sequence listing filed with the application follows.

SEQUENCE LISTING (6 sequences)

SEQ ID NO: 1 - protein, 112 aa, synthetic construct
DVVMTQSPLSLPVTLGQPASISCRSSQSLIYSDGNTRLYWFHQRPGQSPRRLIYGVSNRDSGVPDRFSGSGSGTDFTLKISRVEAEDVGVYYCMQSTHWPHTFGQGTKLEIK

SEQ ID NO: 2 - protein, 125 aa, synthetic construct
QITLKESGPTLVKPTQTLTLTCTFSGFSLSTSGVGVGWIRQPPGEALEWLAVIHWNEANYYSPYLRSRLTITKDTSKNQMVLTVTNMDPVDTATYYCARGANSDSSGRLDAFDIWGQGTMVTVSS

SEQ ID NO: 3 - protein, 111 aa, synthetic construct
QSVLTQPPSASGTPGQTVNISCSGATSNIGGGSVNWYQQLPGAAPRLLIHSDNERASGVPDRFSGSKSGTSASLAISGLQSEDEADYFCASWDDSLDGHVVFGGGTKVTVL

SEQ ID NO: 4 - protein, 121 aa, synthetic construct
QVQLVQSGAELKRPGSSVKVSCRASGDTFKNYAITWVRQAPGQGLEWVGGIDPLVGVPNYTHRFQGRVTITADEPTSTTYMEFRDLTSDDTAVYYCARGVRDQHWSYFDSWGQGTLVTVSS

SEQ ID NO: 5 - protein, 101 aa, synthetic construct
DIELTQSPASLSASVGETVTGNIYSYLAWYQQKQGKSPQLLVYDAKTLADGVPSRFTGSGSGTQFSLKINSLQPEDFGSYYCQHFWNTPRTFGGGTKLEIK

SEQ ID NO: 6 - protein, 117 aa, synthetic construct
GELQESGPELVKPGASVKISCKASGYSFTGYYMNWVKHSPEKSLEWIGEINPSTGGTSYNQKFKAKATLTVDKSSTTAYMQLKGLTSEDSAVYYCASGGYYEGFDYWGQGTTVTVSS